European Patent Specification EP 4 413 152 B1, published August 19, 2026. Title: Direk Karbapenemaz Üçlü (Kpc-2, Oxa-48, Ndm-1) PCR Tanı Kiti. Applicant: TRAKYA UNIVERSITESI REKTORLUGU. Application WO. The sequence listing filed with the application follows.

SEQUENCE LISTING (30 sequences)

SEQ ID NO: 1 - DNA, 21 bp, synthetic construct
  misc_feature 1..21: note = NDM-1 ileri primer
  source 1..21: mol_type = other DNA
tggatcaagcaggagatcaac

SEQ ID NO: 2 - DNA, 19 bp, synthetic construct
  misc_feature 1..19: note = NDM-1 Geri primer
  source 1..19: mol_type = other DNA
atcaggcagccaccaaaag

SEQ ID NO: 3 - DNA, 20 bp, synthetic construct
  misc_feature 1..20: note = KPC-2 leri primer
  source 1..20: mol_type = other DNA
accattcgctaaactcgaac

SEQ ID NO: 4 - DNA, 19 bp, synthetic construct
  misc_feature 1..19: note = KPC-2 Geri primer
  source 1..19: mol_type = other DNA
caatcaacaaactgctgcc

SEQ ID NO: 5 - DNA, 20 bp, synthetic construct
  misc_feature 1..20: note = OXA-48 leri primer
  source 1..20: mol_type = other DNA
agccgcagacaattagccac

SEQ ID NO: 6 - DNA, 22 bp, synthetic construct
  misc_feature 1..22: note = OXA-48 Geri primer
  source 1..22: mol_type = other DNA
cgccaagccatcacaaaagaag

SEQ ID NO: 7 - DNA, 20 bp, synthetic construct
  misc_feature 1..20: note = MCR-1 leri primer
  source 1..20: mol_type = other DNA
ctccaaaatgccctacagac

SEQ ID NO: 8 - DNA, 19 bp, synthetic construct
  misc_feature 1..19: note = MCR-1 Geri primer
  source 1..19: mol_type = other DNA
ataatgactgctgaacgcc

SEQ ID NO: 9 - DNA, 21 bp, synthetic construct
  misc_feature 1..21: note = OXA-23 leri primer
  source 1..21: mol_type = other DNA
aatacagaatatgtgccagcc

SEQ ID NO: 10 - DNA, 19 bp, synthetic construct
  misc_feature 1..19: note = OXA-23 Geri primer
  source 1..19: mol_type = other DNA
ttgcccaaccagtctttcc

SEQ ID NO: 11 - DNA, 21 bp, synthetic construct
  misc_feature 1..21: note = OXA-24 leri primer
  source 1..21: mol_type = other DNA
gcctagagctaatgcagaaag

SEQ ID NO: 12 - DNA, 19 bp, synthetic construct
  misc_feature 1..19: note = OXA-24 Geri primer
  source 1..19: mol_type = other DNA
taacacccattccccatcc

SEQ ID NO: 13 - DNA, 21 bp, synthetic construct
  misc_feature 1..21: note = OXA-58 leri primer
  source 1..21: mol_type = other DNA
gcatttagaccgagcaaaaac

SEQ ID NO: 14 - DNA, 20 bp, synthetic construct
  misc_feature 1..20: note = OXA-58 Geri primer
  source 1..20: mol_type = other DNA
ctctgcgctctacatacaac

SEQ ID NO: 15 - DNA, 20 bp, synthetic construct
  misc_feature 1..20: note = KPIC leri primer
  source 1..20: mol_type = other DNA
ccacactggaactgagacac

SEQ ID NO: 16 - DNA, 20 bp, synthetic construct
  misc_feature 1..20: note = KPIC Geri primer
  source 1..20: mol_type = other DNA
tcacatccgacttgacagac

SEQ ID NO: 17 - DNA, 22 bp, synthetic construct
  misc_feature 1..22: note = Acinetobacter baumannii 16S-rRNA leri primer
  source 1..22: mol_type = other DNA
gggagcaaacaggattagatac

SEQ ID NO: 18 - DNA, 19 bp, synthetic construct
  misc_feature 1..19: note = Acinetobacter baumannii 16S-rRNA Geri primer
  source 1..19: mol_type = other DNA
acccaacatctcacgacac

SEQ ID NO: 19 - DNA, 21 bp, synthetic construct
  misc_feature 1..21: note = IMP leri primer
  source 1..21: mol_type = other DNA
tcattttcatagcgacagcac

SEQ ID NO: 20 - DNA, 19 bp, synthetic construct
  misc_feature 1..19: note = IMP Geri primer
  source 1..19: mol_type = other DNA
tcctttcaggcagccaaac

SEQ ID NO: 21 - DNA, 20 bp, synthetic construct
  misc_feature 1..20: note = VIM leri primer
  source 1..20: mol_type = other DNA
cggagaggacaaagcaagac

SEQ ID NO: 22 - DNA, 20 bp, synthetic construct
  misc_feature 1..20: note = VIM Geri primer
  source 1..20: mol_type = other DNA
attcaatccaccctacccac

SEQ ID NO: 23 - DNA, 20 bp, synthetic construct
  misc_feature 1..20: note = BIC leri primer
  source 1..20: mol_type = other DNA
ttttgactttcgagcggacg

SEQ ID NO: 24 - DNA, 20 bp, synthetic construct
  misc_feature 1..20: note = BIC Geri primer
  source 1..20: mol_type = other DNA
gaagcaaatttgtcgcaccg

SEQ ID NO: 25 - DNA, 20 bp, synthetic construct
  misc_feature 1..20: note = MecA leri primer
  source 1..20: mol_type = other DNA
tggctatcgtgtcacaatcg

SEQ ID NO: 26 - DNA, 20 bp, synthetic construct
  misc_feature 1..20: note = MecA Geri primer
  source 1..20: mol_type = other DNA
acgttgtaaccaccccaaga

SEQ ID NO: 27 - DNA, 20 bp, synthetic construct
  misc_feature 1..20: note = VanA leri primer
  source 1..20: mol_type = other DNA
ttttgactttcgagcggacg

SEQ ID NO: 28 - DNA, 20 bp, synthetic construct
  misc_feature 1..20: note = VanA Geri primer
  source 1..20: mol_type = other DNA
gaagcaaatttgtcgcaccg

SEQ ID NO: 29 - DNA, 20 bp, synthetic construct
  misc_feature 1..20: note = VanB leri primer
  source 1..20: mol_type = other DNA
ggatagctactcccgccttt

SEQ ID NO: 30 - DNA, 20 bp, synthetic construct
  misc_feature 1..20: note = VanB Geri primer
  source 1..20: mol_type = other DNA
ctagacctctacagccgagc